European Patent Application EP 4 206 216 A1, published July 5, 2023. Title: Adeno-associated virus variant capsids and methods of use thereof. Applicant: 4D Molecular Therapeutics, Inc. The sequence listing filed with the application follows.

SEQUENCE LISTING (64 sequences)

SEQ ID NO: 1 - protein, 736 aa, Adeno-associated virus 1
MAADGYLPDWLEDNLSEGIREWWDLKPGAPKPKANQQKQDDGRGLVLPGYKYLGPFNGLDKGEPVNAADAAALEHDKAYDQQLKAGDNPYLRYNHADAEFQERLQEDTSFGGNLGRAVFQAKKRVLEPLGLVEEGAKTAPGKKRPVEQSPQEPDSSSGIGKTGQQPAKKRLNFGQTGDSESVPDPQPLGEPPATPAAVGPTTMASGGGAPMADNNEGADGVGNASGNWHCDSTWLGDRVITTSTRTWALPTYNNHLYKQISSASTGASNDNHYFGYSTPWGYFDFNRFHCHFSPRDWQRLINNNWGFRPKRLNFKLFNIQVKEVTTNDGVTTIANNLTSTVQVFSDSEYQLPYVLGSAHQGCLPPFPADVFMIPQYGYLTLNNGSQAVGRSSFYCLEYFPSQMLRTGNNFTFSYTFEEVPFHSSYAHSQSLDRLMNPLIDQYLYYLNRTQNQSGSAQNKDLLFSRGSPAGMSVQPKNWLPGPCYRQQRVSKTKTDNNNSNFTWTGASKYNLNGRESIINPGTAMASHKDDEDKFFPMSGVMIFGKESAGASNTALDNVMITDEEEIKATNPVATERFGTVAVNFQSSSTDPATGDVHAMGALPGMVWQDRDVYLQGPIWAKIPHTDGHFHPSPLMGGFGLKNPPPQILIKNTPVPANPPAEFSATKFASFITQYSTGQVSVEIEWELQKENSKRWNPEVQYTSNYAKSANVDFTVDNNGLYTEPRPIGTRYLTRPL

SEQ ID NO: 2 - protein, 735 aa, Adeno-associated virus 2 [sequence omitted]

SEQ ID NO: 3 - protein, 736 aa, Adeno-associated virus 3A
MAADGYLPDWLEDNLSEGIREWWALKPGVPQPKANQQHQDNRRGLVLPGYKYLGPGNGLDKGEPVNEADAAALEHDKAYDQQLKAGDNPYLKYNHADAEFQERLQEDTSFGGNLGRAVFQAKKRILEPLGLVEEAAKTAPGKKGAVDQSPQEPDSSSGVGKSGKQPARKRLNFGQTGDSESVPDPQPLGEPPAAPTSLGSNTMASGGGAPMADNNEGADGVGNSSGNWHCDSQWLGDRVITTSTRTWALPTYNNHLYKQISSQSGASNDNHYFGYSTPWGYFDFNRFHCHFSPRDWQRLINNNWGFRPKKLSFKLFNIQVRGVTQNDGTTTIANNLTSTVQVFTDSEYQLPYVLGSAHQGCLPPFPADVFMVPQYGYLTLNNGSQAVGRSSFYCLEYFPSQMLRTGNNFQFSYTFEDVPFHSSYAHSQSLDRLMNPLIDQYLYYLNRTQGTTSGTTNQSRLLFSQAGPQSMSLQARNWLPGPCYRQQRLSKTANDNNNSNFPWTAASKYHLNGRDSLVNPGPAMASHKDDEEKFFPMHGNLIFGKEGTTASNAELDNVMITDEEEIRTTNPVATEQYGTVANNLQSSNTAPTTGTVNHQGALPGMVWQDRDVYLQGPIWAKIPHTDGHFHPSPLMGGFGLKHPPPQIMIKNTPVPANPPTTFSPAKFASFITQYSTGQVSVEIEWELQKENSKRWNPEIQYTSNYNKSVNVDFTVDTNGVYSEPRPIGTRYLTRNL

SEQ ID NO: 4 - protein, 736 aa, Adeno-associated virus 3B
MAADGYLPDWLEDNLSEGIREWWALKPGVPQPKANQQHQDNRRGLVLPGYKYLGPGNGLDKGEPVNEADAAALEHDKAYDQQLKAGDNPYLKYNHADAEFQERLQEDTSFGGNLGRAVFQAKKRILEPLGLVEEAAKTAPGKKRPVDQSPQEPDSSSGVGKSGKQPARKRLNFGQTGDSESVPDPQPLGEPPAAPTSLGSNTMASGGGAPMADNNEGADGVGNSSGNWHCDSQWLGDRVITTSTRTWALPTYNNHLYKQISSQSGASNDNHYFGYSTPWGYFDFNRFHCHFSPRDWQRLINNNWGFRPKKLSFKLFNIQVKEVTQNDGTTTIANNLTSTVQVFTDSEYQLPYVLGSAHQGCLPPFPADVFMVPQYGYLTLNNGSQAVGRSSFYCLEYFPSQMLRTGNNFQFSYTFEDVPFHSSYAHSQSLDRLMNPLIDQYLYYLNRTQGTTSGTTNQSRLLFSQAGPQSMSLQARNWLPGPCYRQQRLSKTANDNNNSNFPWTAASKYHLNGRDSLVNPGPAMASHKDDEEKFFPMHGNLIFGKEGTTASNAELDNVMITDEEEIRTTNPVATEQYGTVANNLQSSNTAPTTRTVNDQGALPGMVWQDRDVYLQGPIWAKIPHTDGHFHPSPLMGGFGLKHPPPQIMIKNTPVPANPPTTFSPAKFASFITQYSTGQVSVEIEWELQKENSKRWNPEIQYTSNYNKSVNVDFTVDTNGVYSEPRPIGTRYLTRNL

SEQ ID NO: 5 - protein, 734 aa, Adeno-associated virus 4
MTDGYLPDWLEDNLSEGVREWWALQPGAPKPKANQQHQDNARGLVLPGYKYLGPGNGLDKGEPVNAADAAALEHDKAYDQQLKAGDNPYLKYNHADAEFQQRLQGDTSFGGNLGRAVFQAKKRVLEPLGLVEQAGETAPGKKRPLIESPQQPDSSTGIGKKGKQPAKKKLVFEDETGAGDGPPEGSTSGAMSDDSEMRAAAGGAAVEGGQGADGVGNASGDWHCDSTWSEGHVTTTSTRTWVLPTYNNHLYKRLGESLQSNTYNGFSTPWGYFDFNRFHCHFSPRDWQRLINNNWGMRPKAMRVKIFNIQVKEVTTSNGETTVANNLTSTVQIFADSSYELPYVMDAGQEGSLPPFPNDVFMVPQYGYCGLVTGNTSQQQTDRNAFYCLEYFPSQMLRTGNNFEITYSFEKVPFHSMYAHSQSLDRLMNPLIDQYLWGLQSTTTGTTLNAGTATTNFTKLRPTNFSNFKKNWLPGPSIKQQGFSKTANQNYKIPATGSDSLIKYETHSTLDGRWSALTPGPPMATAGPADSKFSNSQLIFAGPKQNGNTATVPGTLIFTSEEELAATNATDTDMWGNLPGGDQSNSNLPTVDRLTALGAVPGMVWQNRDIYYQGPIWAKIPHTDGHFHPSPLIGGFGLKHPPPQIFIKNTPVPANPATTFSSTPVNSFITQYSTGQVSVQIDWEIQKERSKRWNPEVQFTSNYGQQNSLLWAPDAAGKYTEPRAIGTRYLTHHL

SEQ ID NO: 6 - protein, 724 aa, Adeno-associated virus 5
MSFVDHPPDWLEEVGEGLREFLGLEAGPPKPKPNQQHQDQARGLVLPGYNYLGPGNGLDRGEPVNRADEVAREHDISYNEQLEAGDNPYLKYNHADAEFQEKLADDTSFGGNLGKAVFQAKKRVLEPFGLVEEGAKTAPTGKRIDDHFPKRKKARTEEDSKPSTSSDAEAGPSGSQQLQIPAQPASSLGADTMSAGGGGPLGDNNQGADGVGNASGDWHCDSTWMGDRVVTKSTRTWVLPSYNNHQYREIKSGSVDGSNANAYFGYSTPWGYFDFNRFHSHWSPRDWQRLINNYWGFRPRSLRVKIFNIQVKEVTVQDSTTTIANNLTSTVQVFTDDDYQLPYVVGNGTEGCLPAFPPQVFTLPQYGYATLNRDNTENPTERSSFFCLEYFPSKMLRTGNNFEFTYNFEEVPFHSSFAPSQNLFKLANPLVDQYLYRFVSTNNTGGVQFNKNLAGRYANTYKNWFPGPMGRTQGWNLGSGVNRASVSAFATTNRMELEGASYQVPPQPNGMTNNLQGSNTYALENTMIFNSQPANPGTTATYLEGNMLITSESETQPVNRVAYNVGGQMATNNQSSTTAPATGTYNLQEIVPGSVWMERDVYLQGPIWAKIPETGAHFHPSPAMGGFGLKHPPPMMLIKNTPVPGNITSFSDVPVSSFITQYSTGQVTVEMEWELKKENSKRWNPEIQYTNNYNDPQFVDFAPDSTGEYRTTRPIGTRYLTRPL

SEQ ID NO: 7 - protein, 736 aa, Adeno-associated virus 6
MAADGYLPDWLEDNLSEGIREWWDLKPGAPKPKANQQKQDDGRGLVLPGYKYLGPFNGLDKGEPVNAADAAALEHDKAYDQQLKAGDNPYLRYNHADAEFQERLQEDTSFGGNLGRAVFQAKKRVLEPFGLVEEGAKTAPGKKRPVEQSPQEPDSSSGIGKTGQQPAKKRLNFGQTGDSESVPDPQPLGEPPATPAAVGPTTMASGGGAPMADNNEGADGVGNASGNWHCDSTWLGDRVITTSTRTWALPTYNNHLYKQISSASTGASNDNHYFGYSTPWGYFDFNRFHCHFSPRDWQRLINNNWGFRPKRLNFKLFNIQVKEVTTNDGVTTIANNLTSTVQVFSDSEYQLPYVLGSAHQGCLPPFPADVFMIPQYGYLTLNNGSQAVGRSSFYCLEYFPSQMLRTGNNFTFSYTFEDVPFHSSYAHSQSLDRLMNPLIDQYLYYLNRTQNQSGSAQNKDLLFSRGSPAGMSVQPKNWLPGPCYRQQRVSKTKTDNNNSNFTWTGASKYNLNGRESIINPGTAMASHKDDKDKFFPMSGVMIFGKESAGASNTALDNVMITDEEEIKATNPVATERFGTVAVNLQSSSTDPATGDVHVMGALPGMVWQDRDVYLQGPIWAKIPHTDGHFHPSPLMGGFGLKHPPPQILIKNTPVPANPPAEFSATKFASFITQYSTGQVSVEIEWELQKENSKRWNPEVQYTSNYAKSANVDFTVDNNGLYTEPRPIGTRYLTRPL

SEQ ID NO: 8 - protein, 737 aa, Adeno-associated virus 7
MAADGYLPDWLEDNLSEGIREWWDLKPGAPKPKANQQKQDNGRGLVLPGYKYLGPFNGLDKGEPVNAADAAALEHDKAYDQQLKAGDNPYLRYNHADAEFQERLQEDTSFGGNLGRAVFQAKKRVLEPLGLVEEGAKTAPAKKRPVEPSPQRSPDSSTGIGKKGQQPARKRLNFGQTGDSESVPDPQPLGEPPAAPSSVGSGTVAAGGGAPMADNNEGADGVGNASGNWHCDSTWLGDRVITTSTRTWALPTYNNHLYKQISSETAGSTNDNTYFGYSTPWGYFDFNRFHCHFSPRDWQRLINNNWGFRPKKLRFKLFNIQVKEVTTNDGVTTIANNLTSTIQVFSDSEYQLPYVLGSAHQGCLPPFPADVFMIPQYGYLTLNNGSQSVGRSSFYCLEYFPSQMLRTGNNFEFSYSFEDVPFHSSYAHSQSLDRLMNPLIDQYLYYLARTQSNPGGTAGNRELQFYQGGPSTMAEQAKNWLPGPCFRQQRVSKTLDQNNNSNFAWTGATKYHLNGRNSLVNPGVAMATHKDDEDRFFPSSGVLIFGKTGATNKTTLENVLMTNEEEIRPTNPVATEEYGIVSSNLQAANTAAQTQVVNNQGALPGMVWQNRDVYLQGPIWAKIPHTDGNFHPSPLMGGFGLKHPPPQILIKNTPVPANPPEVFTPAKFASFITQYSTGQVSVEIEWELQKENSKRWNPEIQYTSNFEKQTGVDFAVDSQGVYSEPRPIGTRYLTRNL

SEQ ID NO: 9 - protein, 738 aa, Adeno-associated virus 8
MAADGYLPDWLEDNLSEGIREWWALKPGAPKPKANQQKQDDGRGLVLPGYKYLGPFNGLDKGEPVNAADAAALEHDKAYDQQLQAGDNPYLRYNHADAEFQERLQEDTSFGGNLGRAVFQAKKRVLEPLGLVEEGAKTAPGKKRPVEPSPQRSPDSSTGIGKKGQQPARKRLNFGQTGDSESVPDPQPLGEPPAAPSGVGPNTMAAGGGAPMADNNEGADGVGSSSGNWHCDSTWLGDRVITTSTRTWALPTYNNHLYKQISNGTSGGATNDNTYFGYSTPWGYFDFNRFHCHFSPRDWQRLINNNWGFRPKRLSFKLFNIQVKEVTQNEGTKTIANNLTSTIQVFTDSEYQLPYVLGSAHQGCLPPFPADVFMIPQYGYLTLNNGSQAVGRSSFYCLEYFPSQMLRTGNNFQFTYTFEDVPFHSSYAHSQSLDRLMNPLIDQYLYYLSRTQTTGGTANTQTLGFSQGGPNTMANQAKNWLPGPCYRQQRVSTTTGQNNNSNFAWTAGTKYHLNGRNSLANPGIAMATHKDDEERFFPSNGILIFGKQNAARDNADYSDVMLTSEEEIKTTNPVATEEYGIVADNLQQQNTAPQIGTVNSQGALPGMVWQNRDVYLQGPIWAKIPHTDGNFHPSPLMGGFGLKHPPPQILIKNTPVPADPPTTFNQSKLNSFITQYSTGQVSVEIEWELQKENSKRWNPEIQYTSNYYKSTSVDFAVNTEGVYSEPRPIGTRYLTRNL

SEQ ID NO: 10 - protein, 736 aa, Adeno-associated virus 9
MAADGYLPDWLEDNLSEGIREWWALKPGAPQPKANQQHQDNARGLVLPGYKYLGPGNGLDKGEPVNAADAAALEHDKAYDQQLKAGDNPYLKYNHADAEFQERLKEDTSFGGNLGRAVFQAKKRLLEPLGLVEEAAKTAPGKKRPVEQSPQEPDSSAGIGKSGAQPAKKRLNFGQTGDTESVPDPQPIGEPPAAPSGVGSLTMASGGGAPVADNNEGADGVGSSSGNWHCDSQWLGDRVITTSTRTWALPTYNNHLYKQISNSTSGGSSNDNAYFGYSTPWGYFDFNRFHCHFSPRDWQRLINNNWGFRPKRLNFKLFNIQVKEVTDNNGVKTIANNLTSTVQVFTDSDYQLPYVLGSAHEGCLPPFPADVFMIPQYGYLTLNDGSQAVGRSSFYCLEYFPSQMLRTGNNFQFSYEFENVPFHSSYAHSQSLDRLMNPLIDQYLYYLSKTINGSGQNQQTLKFSVAGPSNMAVQGRNYIPGPSYRQQRVSTTVTQNNNSEFAWPGASSWALNGRNSLMNPGPAMASHKEGEDRFFPLSGSLIFGKQGTGRDNVDADKVMITNEEEIKTTNPVATESYGQVATNHQSAQAQAQTGWVQNQGILPGMVWQDRDVYLQGPIWAKIPHTDGNFHPSPLMGGFGMKHPPPQILIKNTPVPADPPTAFNKDKLNSFITQYSTGQVSVEIEWELQKENSKRWNPEIQYTSNYYKSNNVEFAVNTEGVYSEPRPIGTRYLTRNL

SEQ ID NO: 11 - protein, 738 aa, Adeno-associated virus 10
MAADGYLPDWLEDNLSEGIREWWDLKPGAPKPKANQQKQDDGRGLVLPGYKYLGPFNGLDKGEPVNAADAAALEHDKAYDQQLKAGDNPYLRYNHADAEFQERLQEDTSFGGNLGRAVFQAKKRVLEPLGLVEEAAKTAPGKKRPVEPSPQRSPDSSTGIGKKGQQPAKKRLNFGQTGESESVPDPQPIGEPPAGPSGLGSGTMAAGGGAPMADNNEGADGVGSSSGNWHCDSTWLGDRVITTSTRTWALPTYNNHLYKQISNGTSGGSTNDNTYFGYSTPWGYFDFNRFHCHFSPRDWQRLINNNWGFRPKRLSFKLFNIQVKEVTQNEGTKTIANNLTSTIQVFTDSEYQLPYVLGSAHQGCLPPFPADVFMIPQYGYLTLNNGSQAVGRSSFYCLEYFPSQMLRTGNNFEFSYTFEDVPFHSSYAHSQSLDRLMNPLIDQYLYYLSRTQSTGGTQGTQQLLFSQAGPANMSAQAKNWLPGPCYRQQRVSTTLSQNNNSNFAWTGATKYHLNGRDSLVNPGVAMATHKDDEERFFPSSGVLMFGKQGAGRDNVDYSSVMLTSEEEIKTTNPVATEQYGVVADNLQQANTGPIVGNVNSQGALPGMVWQNRDVYLQGPIWAKIPHTDGNFHPSPLMGGFGLKHPPPQILIKNTPVPADPPTTFSQAKLASFITQYSTGQVSVEIEWELQKENSKRWNPEIQYTSNYYKSTNVDFAVNTEGTYSEPRPIGTRYLTRNL

SEQ ID NO: 12 - protein, 738 aa, Adeno-associated virus rh10
MAADGYLPDWLEDNLSEGIREWWALKPGAPKPKANQQKQDDGRGLVLPGYKYLGPFNGLDKGEPVNAADAAALEHDKAYDQQLKAGDNPYLRYNHADAEFQERLQEDTSFGGNLGRAVFQAKKRVLEPLGLVEEGAKTAPGKKRPVEPSPQRSPDSSTGIGKKGQQPAKKRLNFGQTGDSESVPDPQPIGEPPAGPSGLGSGTMAAGGGAPMADNNEGADGVGSSSGNWHCDSTWLGDGVITTSTRTWALPTYNNHLYKQISNGTSGGSTNDNTYFGYSTPWGYFDFNRFHCHFSPRDWQRLINNNWGFRPKSLNFKLFNIQVKEVTQNEGTKTIANNLTSTIQVFTDSEYQLPYVLGSAHQGCLPPFPADVFMIPQYGYLTLNNGSQAVGRSSFYCLEYFPSQMLRTGNNFEFSYQFEDVPFHSSYAHSQSLDRLMNPLIDQYLYYLSRTQSTGGTAGTQQLLFSQAGPNNMSAQAKNWLPGPCYRQQRVSTTLSQNDNSNFAWTGATKYHLNGRDSLVNPGVAMATHKDDEERFFPSSGVLMFGKQGAGKDNVDYSSVMLTSEEEIKTTNPVATEQYGVVADNLQQQNAAPIVGAVNSQGALPGMVWQNRDVYLQGPIWAKIPHTDGNFHPSPLMGGFGLKHPPPQILIKNTPVPADPPTTFSQAKLASFITQYSTGQVSVEIEWELQKENSKRWNPEIQYTSNYYKSTNVDFAVNTDGTYSEPRPIGTRYLTRNL

SEQ ID NO: 13 - protein, 7 aa, synthetic construct
  REGION 1..7: note = heterologous peptide insertion
QADTTKN

SEQ ID NO: 14 - protein, 7 aa, synthetic construct
  REGION 1..7: note = heterologous peptide insertion
ISDQTKH

SEQ ID NO: 15 - protein, 7 aa, synthetic construct
  REGION 1..7: note = heterologous peptide insertion
ASDSTKA

SEQ ID NO: 16 - protein, 7 aa, synthetic construct
  REGION 1..7: note = heterologous peptide insertion
NQDYTKT

SEQ ID NO: 17 - protein, 7 aa, synthetic construct
  REGION 1..7: note = heterologous peptide insertion
HDITKNI

SEQ ID NO: 18 - protein, 7 aa, synthetic construct
  REGION 1..7: note = heterologous peptide insertion
HPDTTKN

SEQ ID NO: 19 - protein, 7 aa, synthetic construct
  REGION 1..7: note = heterologous peptide insertion
HQDTTKN

SEQ ID NO: 20 - protein, 7 aa, synthetic construct
  REGION 1..7: note = heterologous peptide insertion
NKTTNKD

SEQ ID NO: 21 - protein, 7 aa, synthetic construct
  REGION 1..7: note = heterologous peptide insertion
ISNENEH

SEQ ID NO: 22 - protein, 7 aa, synthetic construct
  REGION 1..7: note = heterologous peptide insertion
QANANEN

SEQ ID NO: 23 - protein, 7 aa, synthetic construct
  REGION 1..7: note = heterologous peptide insertion
GKSKVID

SEQ ID NO: 24 - protein, 7 aa, synthetic construct
  REGION 1..7: note = heterologous peptide insertion
TNRTSPD

SEQ ID NO: 25 - protein, 7 aa, synthetic construct
  REGION 1..7: note = heterologous peptide insertion
PNSTHGS

SEQ ID NO: 26 - protein, 7 aa, synthetic construct
  REGION 1..7: note = heterologous peptide insertion
KDRAPST

SEQ ID NO: 27 - protein, 10 aa, synthetic construct
  REGION 1..10: note = heterologous peptide insertion
LAQADTTKNA

SEQ ID NO: 28 - protein, 10 aa, synthetic construct
  REGION 1..10: note = heterologous peptide insertion
LAISDQTKHA

SEQ ID NO: 29 - protein, 10 aa, synthetic construct
  REGION 1..10: note = heterologous peptide insertion
LGISDQTKHA

SEQ ID NO: 30 - protein, 10 aa, synthetic construct
  REGION 1..10: note = heterologous peptide insertion
LAASDSTKAA

SEQ ID NO: 31 - protein, 10 aa, synthetic construct
  REGION 1..10: note = heterologous peptide insertion
LANQDYTKTA

SEQ ID NO: 32 - protein, 10 aa, synthetic construct
  REGION 1..10: note = heterologous peptide insertion
LAHDITKNIA

SEQ ID NO: 33 - protein, 10 aa, synthetic construct
  REGION 1..10: note = heterologous peptide insertion
LAHPDTTKNA

SEQ ID NO: 34 - protein, 10 aa, synthetic construct
  REGION 1..10: note = heterologous peptide insertion
LAHQDTTKNA

SEQ ID NO: 35 - protein, 10 aa, synthetic construct
  REGION 1..10: note = heterologous peptide insertion
LANKTTNKDA

SEQ ID NO: 36 - protein, 10 aa, synthetic construct
  REGION 1..10: note = heterologous peptide insertion
LPISNENEHA

SEQ ID NO: 37 - protein, 10 aa, synthetic construct
  REGION 1..10: note = heterologous peptide insertion
LPQANANENA

SEQ ID NO: 38 - protein, 10 aa, synthetic construct
  REGION 1..10: note = heterologous peptide insertion
LAGKSKVIDA

SEQ ID NO: 39 - protein, 10 aa, synthetic construct
  REGION 1..10: note = heterologous peptide insertion
LATNRTSPDA

SEQ ID NO: 40 - protein, 10 aa, synthetic construct
  REGION 1..10: note = heterologous peptide insertion
LAPNSTHGSA

SEQ ID NO: 41 - protein, 10 aa, synthetic construct
  REGION 1..10: note = heterologous peptide insertion
LAKDRAPSTA

SEQ ID NO: 42 - protein, 745 aa, synthetic construct
  REGION 1..745: note = Variant AAV capsid
MAADGYLPDWLEDTLSEGIRQWWKLKPGPPPPKAAERHKDDSRGLVLPGYKYLGPFNGLDKGEPVNEADAAALEHDKAYDRQLDSGDNPYLKYNHADAEFQERLKEDTSFGGNLGRAVFQAKKRVLEPLGLVEEPVKTAPGKKRPVEHSPVEPDSSSGTGKAGQQPARKRLNFGQTGDADSVPDPQPLGQPPAAPSGLGTNTMATGSGAPMADNNEGADGVGNSSGNWHCDSTWMGDRVITTSTRTWALPTYNNHLYKQISSQSGASNDNHYFGYSTPWGYFDFNRFHCHFSPRDWQRLINNNWGFRPKRLNFKLFNIQVKEVTQNDGTTTIANNLTSTVQVFTDSEYQLPYVLGSAHQGCLPPFPADVFMVPQYGYLTLNNGSQAVGRSSFYCLEYFPSQMLRTGNNFTFSYTFEDVPFHSSYAHSQSLDRLMNPLIDQYLYYLSRTNTPSGTTTQSRLQFSQAGASDIRDQSRNWLPGPCYRQQRVSKTSADNNNSEYSWTGATKYHLNGRDSLVNPGPAMASHKDDEEKFFPQSGVLIFGKQGSEKTNVDIEKVMITDEEEIRTTNPVATEQYGSVSTNLQRGNLAISDQTKHARQAATADVNTQGVLPGMVWQDRDVYLQGPIWAKIPHTDGHFHPSPLMGGFGLKHPPPQILIKNTPVPANPSTTFSAAKFASFITQYSTGQVSVEIEWELQKENSKRWNPEIQYTSNYNKSVNVDFTVDTNGVYSEPRPIGTRYLTRNL

SEQ ID NO: 43 - protein, 745 aa, synthetic construct
  REGION 1..745: note = AAV capsid variant
MAADGYLPDWLEDTLSEGIRQWWKLKPGPPPPKPAERHKDDSRGLVLPGYKYLGPFNGLDKGEPVNEADAAALEHDKAYDRQLDSGDNPYLKYNHADAEFQERLKEDTSFGGNLGRAVFQAKKRVLEPLGLVEEPVKTAPGKKRPVEHSPVEPDSSSGTGKAGQQPARKRLNFGQTGDADSVPDPQPLGQPPAAPSGLGTNTMATGSGAPMADNNEGADGVGNSSGNWHCDSTWMGDRVITTSTRTWALPTYNNHLYKQISSQSGASNDNHYFGYSTPWGYFDFNRFHCHFSPRDWQRLINNNWGFRPKRLKFKLFNIQVKEVTQNDGTTTIANNLTSTVQVFTDSEYQLPYVLGSAHQGCLPPFPADVFMVPQYGYLTLNNGSQAVGRSSFYCLEYFPSQMLRTGNNFTFSYTFEDVPFHSSYAHSQSLDRLMNPLIDQYLYYLSRTDTPSGTTTQSRLQFSQAGASDIRNQSRNWLPGPCYRQQRVSKTSADNNNSEYSWTGATKYHLNGRDSLVNPGPAMASHKDDEEKFFPQSGVLIFGKQGSEKTSVDIEKVMITDEEEIRTTNPVATEQYGSVSTNLQRGNLAISDQTKHARQAATADVNTQGVLPGMVWQDRDVYLQGPIWAKIPHTDGHFHPSPLMGGFGLKHPPPQILIKNTPVPANPSTTFSAAKFASFITQYSTGQVSVEIEWELQKENSKRWNPEVQYTSNYNKSVNVDFTVDTNGVYSEPRPIGTRYLTRNQ

SEQ ID NO: 44 - protein, 745 aa, synthetic construct
  REGION 1..745: note = AAV capsid variant
MAADGYLPDWLEDTLSEGIRQWWKLKPGPPPPKPAERHKDDSRGLVLPGYKYLGPFNGLDKGEPVNEADAAALEHDKAYDRQLDSGDNPYLKYNHADAEFQERLKEDTSFGGNLGRAVFQAKKRVLEPLGLVEEPVKTAPGKKRPVEHSPVEPDSSSGTGKAGQQPARKRLNFGQTGDADSVPDPQPLGQPPAAPSGLGTNTMATGSGAPMADNNEGADGVGNSSGNWHCDSTWMGDRVITTSTRTWALPTYNNHLYKQISSQSGASNDNHYFGYSTPWGYFDFNRFHCHFSPRDWQRLINNNWGFRPKRLNFKLFNIQVKEVTQNDGTTTIANNLTSTVQVFTDSEYQLPYVLGSAHQGCLPPFPADVFMVPQYGYLTLNNGSQAVGRSSFYCLEYFPSQMLRTGNNFTFSYTFEDVPFHSSYAHSQSLDRLMNPLIDQYLYYLSRTNTPSGTTTQSRLQFSQAGASDIRDQSRNWLPGPCYRQQRVSKTSADNNNSEYSWTGATKYHLNGRDSLVNPGPAMASHKDDEEKFFPQSGVLIFGKQGSEKTNVDIEKVMITDEEEIRTTNPVATEQYGSVSTNLQRGNLGISDQTKHARQAATADVNTQGVLPGMVWQDRDVYLQGPIWAKIPHTDGHFHPSPLMGGFGLKHPPPQILIKNTPVPANPSTTFSAAKFASFITQYSTGQVSVEIEWELQKENSKRWNPEIQYTSNYNKSVNVDFTVDTNGVYSEPRPIGTRYLTRNL

SEQ ID NO: 45 - protein, 745 aa, synthetic construct
  REGION 1..745: note = AAV capsid variant
MAADGYLPDWLEDTLSEGIRQWWKLKPGPPPPKPAERHKDDSRGLVLPGYKYLGPFNGLDKGEPVNEADAAALEHDKAYDRQLDSGDNPYLKYNHADAEFQERLKEDTSFGGNLGRAVFQAKKRVLEPLGLVEEPVKTAPGKKRPVEHSPVEPDSSSGTGKAGQQPARKRLNFGQTGDADSVPDPQPLGQPPAAPSGLGTNTMATGSGAPMADNNEGADGVGNSSGNWHCDSTWMGDRVITTSTRTWALPTYNNHLYKQISSQSGASNDNHYFGYSTPWGYFDFNRFHCHFSPRDWQRLINNNWGFRPKRLNFKLFNIQVKEVTQNDGTTTIANNLTSTVQVFTDSEYQLPYVLGSAHQGCLPPFPADVFMVPQYGYLTLNNGSQAVGRSSFYCLEYFPSQMLRTGNNFTFSYTFEDVPFHSSYAHSQSLDRLMNPLIDQYLYYLSRTNTPSGTTTQSRLQFSQAGASDIRDQSRNWLPGPCYRQQRVSKTSADNNNSEYSWTGATKYHLNGRDSLVNPGPAMASHKDDEEKFFPQSGVLIFGKQGSEKTNVDIEKVMITDEEEIRTTNPVATEQYGSVSTNLQRGNLAQADTTKNARQAATADVNTQGVLPGMVWQDRDVYLQGPIWAKIPHTDGHFHPSPLMGGFGLKHPPPQILIKNTPVPANPSTTFSAAKFASFITQYSTGQVSVEIEWELQKENSKRWNPEVQYTSNYNKSVNVDFTVDTNGVYSEPRPIGTRYLTRNL

SEQ ID NO: 46 - protein, 745 aa, synthetic construct
  REGION 1..745: note = AAV capsid variant
MAADGYLPDWLEDTLSEGIRQWWKLKPGPPPPKPAERHKDDSRGLVLPGYKYLGPFNGLDKGEPVNEADAAALEHDKAYDRQLDSGDNPYLKYNHADAEFQERLKEDTSFGGNLGRAVFQAKKRVLEPLGLVEEPVKTAPGKKRPVEHSPVEPDSSSGTGKAGQQPARKRLNFGQTGDADSVPDPQPLGQPPAAPSGLGTNTMATGSGAPMADNNEGADGVGNSSGNWHCDSTWMGDRVITTSTRTWALPTYNNHLYKQISSQSGASNDNHYFGYSTPWGYFDFNRFHCHFSPRDWQRLINNNWGFRPKRLNFKLFNIQVKEVTQNDGTTTIANNLTSTVQVFTDSEYQLPYVLGSAHQGCLPPFPADVFMVPQYGYLTLNNGSQAVGRSSFYCLEYFPSQMLRTGNNFTFSYTFEDVPFHSSYAHSQSLDRLMNPLIDQYLYYLSRTNTPSGTTTQSRLQFSQAGASDIRDQSRNWLPGPCYRQQRVSKTSADNNNSEYSWTGATKYHLNGRDSLVNPGPAMASHKDDEEKFFPQSGVLIFGKQGSEKTNVDIEKVMITDEEEIRTTNPVATEQYGSVSTNLQRGNLAHDITKNIARQAATADVNTQGVLPGMVWQDRDVYLQGPIWAKIPHTDGHFHPSPLMGGFGLKHPPPQILIKNTPVPANPSTTFSAAKFASFITQYSTGQVSVEIEWELQKENSKRWNPEIQYTSNYNKSVNVDFTVDTNGVYSEPRPIGTRYLTRNL

SEQ ID NO: 47 - protein, 745 aa, synthetic construct
  REGION 1..745: note = AAV capsid variant
MAADGYLPDWLEDTLSEGIRQWWKLKPGPPPPKPAERHKDDSRGLVLPGYKYLGPFNGLDKGEPVNEADAAALEHDKAYDRQLDSGDNPYLKYNHADAEFQERLKEDTSFGGNLGRAVFQAKKRVLEPLGLVEEPVKTAPGKKRPVEHSPVEPDSSSGTGKAGQQPARKRLNFGQTGDADSVPDPQPLGQPPAAPSGLGTNTMATGSGAPMADNNEGADGVGNSSGNWHCDSTWMGDRVITTSTRTWALPTYNNHLYKQISSQSGASNDNHYFGYSTPWGYFDFNRFHCHFSPRDWQRLINNNWGFRPKRLNFKLFNIQVKEVTQNDGTTTIANNLTSTVQVFTDSEYQLPYVLGSAHQGCLPPFPADVFMVPQYGYLTLNNGSQAVGRSSFYCLEYFPSQMLRTGNNFTFSYTFEDVPFHSSYAHSQSLDRLMNPLIDQYLYYLSRTNTPSGTTTQSRLQFSQAGASDIRDQSRNWLPGPCYRQQRVSKTSADNNNSEYSWTGATKYHLNGRDSLVNPGPAMASHKDDEEKFFPQSGVLIFGKQGSEKTNVDIEKVMITDEEEIRTTNPVATEQYGSVSTNLQRGNLANQDYTKTARQAATADVNTQGVLPGMVWQDRDVYLQGPIWAKIPHTDGHFHPSPLMGGFGLKHPPPQILIKNTPVPANPSTTFSAAKFASFITQYSTGQVSVEIEWELQKENSKRWNPEIQYTSNYNKSVNVDFTVDTNGVYSEPRPIGTRYLTRNL

SEQ ID NO: 48 - protein, 745 aa, synthetic construct
  REGION 1..745: note = AAV capsid variant
MAADGYLPDWLEDTLSEGIRQWWKLKPGPPPPKPAERHKDDSRGLVLPGYKYLGPFNGLDKGEPVNEADAAALEHDKAYDRQLDSGDNPYLKYNHADAEFQERLKEDTSFGGNLGRAVFQAKKRVLEPLGLVEEPVKTAPGKKRPVEHSPVEPDSSSGTGKAGQQPARKRLNFGQTGDADSVPDPQPLGQPPAAPSGLGTNTMATGSGAPMADNNEGADGVGNSSGNWHCDSTWMGDRVITTSTRTWALPTYNNHLYKQISSQSGASNDNHYFGYSTPWGYFDFNRFHCHFSPRDWQRLINNNWGFRPKRLNFKLFNIQVKEVTQNDGTTTIANNLTSTVQVFTDSEYQLPYVLGSAHQGCLPPFPADVFMVPQYGYLTLNNGSQAVGRSSFYCLEYFPSQMLRTGNNFTFSYTFEDVPFHSSYAHSQSLDRLMNPLIDQYLYYLSRTNTPSGTTTQSRLQFSQAGASDIRDQSRNWLPGPCYRQQRVSKTSADNNNSEYSWTGATKYHLNGRDSLVNPGPAMASHKDDEEKFFPQSGVLIFGKQGSEKTNVDIEKVMITDEEEIRTTNPVATEQYGSVSTNLQRGNLAPNSTHGSARQAATADVNTQGVLPGMVWQDRDVYLQGPIWAKIPHTDGHFHPSPLMGGFGLKHPPPQILIKNTPVPANPSTTFSAAKFASFITQYSTGQVSVEIEWELQKENSKRWNPEIQYTSNYNKSVNVDFTVDTNGVYSEPRPIGTRYLTRNL

SEQ ID NO: 49 - protein, 745 aa, synthetic construct
  REGION 1..745: note = AAV capsid variant
MAADGYLPDWLEDTLSEGIRQWWKLKPGPPPPKPAERHKDDSRGLVLPGYKYLGPFNGLDKGEPVNEADAAALEHDKAYDRQLDSGDNPYLKYNHADAEFQERLKEDTSFGGNLGRAVFQAKKRVLEPLGLVEEPVKTAPGKKRPVEHSPVEPDSSSGTGKAGQQPARKRLNFGQTGDADSVPDPQPLGQPPAAPSGLGTNTMATGSGAPMADNNEGADGVGNSSGNWHCDSTWMGDRVITTSTRTWALPTYNNHLYKQISSQSGASNDNHYFGYSTPWGYFDFNRFHCHFSPRDWQRLINNNWGFRPKRLNFKLFNIQVKEVTQNDGTTTIANNLTSTVQVFTDSEYQLPYVLGSAHQGCLPPFPADVFMVPQYGYLTLNNGSQAVGRSSFYCLEYFPSQMLRTGNNFTFSYTFEDVPFHSSYAHSQSLDRLMNPLIDQYLYYLSRTNTPSGTTTQSRLQFSQAGASDIRDQSRNWLPGPCYRQQRVSKTSADNNNSEYSWTGATKYHLNGRDSLVNPGPAMASHKDDEEKFFPQSGVLIFGKQGSEKTNVDIEKVMITDEEEIRTTNPVATEQYGSVSTNLQRGNLANKTTNKDARQAATADVNTQGVLPGMVWQDRDVYLQGPIWAKIPHTDGHFHPSPLMGGFGLKHPPPQILIKNTPVPANPSTTFSAAKFASFITQYSTGQVSVEIEWELQKENSKRWNPEIQYTSNYNKSVNVDFTVDTNGVYSEPRPIGTRYLTRNL

SEQ ID NO: 50 - protein, 745 aa, synthetic construct
  REGION 1..745: note = AAV capsid variant
MAADGYLPDWLEDTLSEGIRQWWKLKPGPPPPKPAERHKDDSRGLVLPGYKYLGPFNGLDKGEPVNEADAAALEHDKAYDRQLDSGDNPYLKYNHADAEFQERLKEDTSFGGNLGRAVFQAKKRVLEPLGLVEEPVKTAPGKKRPVEHSPVEPDSSSGTGKAGQQPARKRLNFGQTGDADSVPDPQPLGQPPAAPSGLGTNTMATGSGAPMADNNEGADGVGNSSGNWHCDSTWMGDRVITTSTRTWALPTYNNHLYKQISSQSGASNDNHYFGYSTPWGYFDFNRFHCHFSPRDWQRLINNNWGFRPKRLNFKLFNIQVKEVTQNDGTTTIANNLTSTVQVFTDSEYQLPYVLGSAHQGCLPPFPADVFMVPQYGYLTLNNGSQAVGRSSFYCLEYFPSQMLRTGNNFTFSYTFEDVPFHSSYAHSQSLDRLMNPLIDQYLYYLSRTNTPSGTTTQSRLQFSQAGASDIRDQSRNWLPGPCYRQQRVSKTSADNNNSEYSWTGATKYHLNGRDSLVNPGPAMASHKDDEEKFFPQSGVLIFGKQGSEKTNVDIEKVMITDEEEIRTTNPVATEQYGSVSTNLQRGNLATNRTSPDARQAATADVNTQGVLPGMVWQDRDVYLQGPIWAKIPHTDGHFHPSPLMGGFGLKHPPPQILIKNTPVPANPSTTFSAAKFASFITQYSTGQVSVEIEWELQKENSKRWNPEIQYTSNYNKSVNVDFTVDTNGVYSEPRPIGTRYLTRNL

SEQ ID NO: 51 - protein, 745 aa, synthetic construct
  REGION 1..745: note = AAV capsid variant
MAADGYLPDWLEDTLSEGIRQWWKLKPGPPPPKPAERHKDDSRGLVLPGYKYLGPFNGLDKGEPVNEADAAALEHDKAYDRQLDSGDNPYLKYNHADAEFQERLKEDTSFGGNLGRAVFQAKKRVLEPLGLVEEPVKTAPGKKRPVEHSPVEPDSSSGTGKAGQQPARKRLNFGQTGDADSVPDPQPLGQPPAAPSGLGTNTMATGSGAPMADNNEGADGVGNSSGNWHCDSTWMGDRVITTSTRTWALPTYNNHLYKQISSQSGASNDNHYFGYSTPWGYFDFNRFHCHFSPRDWQRLINNNWGFRPKRLNFKLFNIQVKEVTQNDGTTTIANNLTSTVQVFTDSEYQLPYVLGSAHQGCLPPFPADVFMVPQYGYLTLNNGSQAVGRSSFYCLEYFPSQMLRTGNNFTFSYTFEDVPFHSSYAHSQSLDRLMNPLIDQYLYYLSRTNTPSGTTTQSRLQFSQAGASDIRDQSRNWLPGPCYRQQRVSKTSADNNNSEYSWTGATKYHLNGRDSLVNPGPAMASHKDDEEKFFPQSGVLIFGKQGSEKTNVDIEKVMITDEEEIRTTNPVATEQYGSVSTNLQRGNLAGKSKVIDARQAATADVNTQGVLPGMVWQDRDVYLQGPIWAKIPHTDGHFHPSPLMGGFGLKHPPPQILIKNTPVPANPSTTFSAAKFASFITQYSTGQVSVEIEWELQKENSKRWNPEIQYTSNYNKSVNVDFTVDTNGVYSEPRPIGTRYLTRNL

SEQ ID NO: 52 - protein, 745 aa, synthetic construct
  REGION 1..745: note = AAV capsid variant
MAADGYLPDWLEDTLSEGIRQWWKLKPGPPPPKPAERHKDDSRGLVLPGYKYLGPFNGLDKGEPVNEADAAALEHDKAYDRQLDSGDNPYLKYNHADAEFQERLKEDTSFGGNLGRAVFQAKKRVLEPLGLVEEPVKTAPGKKRPVEHSPVEPDSSSGTGKAGQQPARKRLNFGQTGDADSVPDPQPLGQPPAAPSGLGTNTMATGSGAPMADNNEGADGVGNSSGNWHCDSTWMGDRVITTSTRTWALPTYNNHLYKQISSQSGASNDNHYFGYSTPWGYFDFNRFHCHFSPRDWQRLINNNWGFRPKRLNFKLFNIQVKEVTQNDGTTTIANNLTSTVQVFTDSEYQLPYVLGSAHQGCLPPFPADVFMVPQYGYLTLNNGSQAVGRSSFYCLEYFPSQMLRTGNNFTFSYTFEDVPFHSSYAHSQSLDRLMNPLIDQYLYYLSRTNTPSGTTTQSRLQFSQAGASDIRDQSRNWLPGPCYRQQRVSKTSADNNNSEYSWTGATKYHLNGRDSLVNPGPAMASHKDDEEKFFPQSGVLIFGKQGSEKTNVDIEKVMITDEEEIRTTNPVATEQYGSVSTNLQRGNLAASDSTKAARQAATADVNTQGVLPGMVWQDRDVYLQGPIWAKIPHTDGHFHPSPLMGGFGLKHPPPQILIKNTPVPANPSTTFSAAKFASFITQYSTGQVSVEIEWELQKENSKRWNPEIQYTSNYNKSVNVDFTVDTNGVYSEPRPIGTRYLTRNL

SEQ ID NO: 53 - protein, 745 aa, synthetic construct
  REGION 1..745: note = AAV capsid variant
MAADGYLPDWLEDTLSEGIRQWWKLKPGPPPPKPAERHKDDSRGLVLPGYKYLGPFNGLDKGEPVNEADAAALEHDKAYDRQLDSGDNPYLKYNHADAEFQERLKEDTSFGGNLGRAVFQAKKRVLEPLGLVEEPVKTAPGKKRPVEHSPVEPDSSSGTGKAGQQPARKRLNFGQTGDADSVPDPQPLGQPPAAPSGLGTNTMATGSGAPMADNNEGADGVGNSSGNWHCDSTWMGDRVITTSTRTWALPTYNNHLYKQISSQSGASNDNHYFGYSTPWGYFDFNRFHCHFSPRDWQRLINNNWGFRPKRLNFKLFNIQVKEVTQNDGTTTIANNLTSTVQVFTDSEYQLPYVLGSAHQGCLPPFPADVFMVPQYGYLTLNNGSQAVGRSSFYCLEYFPSQMLRTGNNFTFSYTFEDVPFHSSYAHSQSLDRLMNPLIDQYLYYLSRTNTPSGTTTQSRLQFSQAGASDIRDQSRNWLPGPCYRQQRVSKTSADNNNSEYSWTGATKYHLNGRDSLVNPGPAMASHKDDEEKFFPQSGVLIFGKQGSEKTNVDIEKVMITDEEEIRTTNPVATEQYGSVSTNLQRGNLAKDRAPSTARQAATADVNTQGVLPGMVWQDRDVYLQGPIWAKIPHTDGHFHPSPLMGGFGLKHPPPQILIKNTPVPANPSTTFSAAKFASFITQYSTGQVSVEIEWELQKENSKRWNPEIQYTSNYNKSVNVDFTVDTNGVYSEPRPIGTRYLTRNL

SEQ ID NO: 54 - protein, 745 aa, synthetic construct
  REGION 1..745: note = AAV capsid variant
MAADGYLPDWLEDTLSEGIRQWWKLKPGPPPPKPAERHKDDSRGLVLPGYKYLGPFNGLDKGEPVNEADAAALEHDKAYDRQLDSGDNPYLKYNHADAEFQERLKEDTSFGGNLGRAVFQAKKRVLEPLGLVEEPVKTAPGKKRPVEHSPVEPDSSSGTGKAGQQPARKRLNFGQTGDADSVPDPQPLGQPPAAPSGLGTNTMATGSGAPMADNNEGADGVGNSSGNWHCDSTWMGDRVITTSTRTWALPTYNNHLYKQISSQSGASNDNHYFGYSTPWGYFDFNRFHCHFSPRDWQRLINNNWGFRPKRLNFKLFNIQVKEVTQNDGTTTIANNLTSTVQVFTDSEYQLPYVLGSAHQGCLPPFPADVFMVPQYGYLTLNNGSQAVGRSSFYCLEYFPSQMLRTGNNFTFSYTFEDVPFHSSYAHSQSLDRLMNPLIDQYLYYLSRTNTPSGTTTQSRLQFSQAGASDIRDQSRNWLPGPCYRQQRVSKTSADNNNSEYSWTGATKYHLNGRDSLVNPGPAMASHKDDEEKFFPQSGVLIFGKQGSEKTNVDIEKVMITDEEEIRTTNPVATEQYGSVSTNLQRGNLAHQDTTKNARQAATADVNTQGVLPGMVWQDRDVYLQGPIWAKIPHTDGHFHPSPLMGGFGLKHPPPQILIKNTPVPANPSTTFSAAKFASFITQYSTGQVSVEIEWELQKENSKRWNPEIQYTSNYNKSVNVDFTVDTNGVYSEPRPIGTRYLTRNL

SEQ ID NO: 55 - protein, 745 aa, synthetic construct
  REGION 1..745: note = AAV capsid variant
MAADGYLPDWLEDTLSEGIRQWWKLKPGPPPPKPAERHKDDSRGLVLPGYKYLGPFNGLDKGEPVNEADAAALEHDKAYDRQLDSGDNPYLKYNHADAEFQERLKEDTSFGGNLGRAVFQAKKRVLEPLGLVEEPVKTAPGKKRPVEHSPVEPDSSSGTGKAGQQPARKRLNFGQTGDADSVPDPQPLGQPPAAPSGLGTNTMATGSGAPMADNNEGADGVGNSSGNWHCDSTWMGDRVITTSTRTWALPTYNNHLYKQISSQSGASNDNHYFGYSTPWGYFDFNRFHCHFSPRDWQRLINNNWGFRPKRLNFKLFNIQVKEVTQNDGTTTIANNLTSTVQVFTDSEYQLPYVLGSAHQGCLPPFPADVFMVPQYGYLTLNNGSQAVGRSSFYCLEYFPSQMLRTGNNFTFSYTFEDVPFHSSYAHSQSLDRLMNPLIDQYLYYLSRTNTPSGTTTQSRLQFSQAGASDIRDQSRNWLPGPCYRQQRVSKTSADNNNSEYSWTGATKYHLNGRDSLVNPGPAMASHKDDEEKFFPQSGVLIFGKQGSEKTNVDIEKVMITDEEEIRTTNPVATEQYGSVSTNLQRGNLPISNENEHARQAATADVNTQGVLPGMVWQDRDVYLQGPIWAKIPHTDGHFHPSPLMGGFGLKHPPPQILIKNTPVPANPSTTFSAAKFASFITQYSTGQVSVEIEWELQKENSKRWNPEIQYTSNYNKSVNVDFTVDTNGVYSEPRPIGTRYLTRNL

SEQ ID NO: 56 - protein, 745 aa, synthetic construct
  REGION 1..745: note = AAV capsid variant
MAADGYLPDWLEDTLSEGIRQWWKLKPGPPPPKPAERHKDDSRGLVLPGYKYLGPFNGLDKGEPVNEADAAALEHDKAYDRQLDSGDNPYLKYNHADAEFQERLKEDTSFGGNLGRAVFQAKKRVLEPLGLVEEPVKTAPGKKRPVEHSPVEPDSSSGTGKAGQQPARKRLNFGQTGDADSVPDPQPLGQPPAAPSGLGTNTMATGSGAPMADNNEGADGVGNSSGNWHCDSTWMGDRVITTSTRTWALPTYNNHLYKQISSQSGASNDNHYFGYSTPWGYFDFNRFHCHFSPRDWQRLINNNWGFRPKRLNFKLFNIQVKEVTQNDGTTTIANNLTSTVQVFTDSEYQLPYVLGSAHQGCLPPFPADVFMVPQYGYLTLNNGSQAVGRSSFYCLEYFPSQMLRTGNNFTFSYTFEDVPFHSSYAHSQSLDRLMNPLIDQYLYYLSRTNTPSGTTTQSRLQFSQAGASDIRDQSRNWLPGPCYRQQRVSKTSADNNNSEYSWTGATKYHLNGRDSLVNPGPAMASHKDDEEKFFPQSGVLIFGKQGSEKTNVDIEKVMITDEEEIRTTNPVATEQYGSVSTNLQRGNLPQANANENARQAATADVNTQGVLPGMVWQDRDVYLQGPIWAKIPHTDGHFHPSPLMGGFGLKHPPPQILIKNTPVPANPSTTFSAAKFASFITQYSTGQVSVEIEWELQKENSKRWNPEIQYTSNYNKSVNVDFTVDTNGVYSEPRPIGTRYLTRNL

SEQ ID NO: 57 - protein, 745 aa, synthetic construct
  REGION 1..745: note = AAV capsid variant
MAADGYLPDWLEDTLSEGIRQWWKLKPGPPPPKPAERHKDDSRGLVLPGYKYLGPFNGLDKGEPVNEADAAALEHDKAYDRQLDSGDNPYLKYNHADAEFQERLKEDTSFGGNLGRAVFQAKKRVLEPLGLVEEPVKTAPGKKRPVEHSPVEPDSSSGTGKAGQQPARKRLNFGQTGDADSVPDPQPLGQPPAAPSGLGTNTMATGSGAPMADNNEGADGVGNSSGNWHCDSTWMGDRVITTSTRTWALPTYNNHLYKQISSQSGASNDNHYFGYSTPWGYFDFNRFHCHFSPRDWQRLINNNWGFRPKRLNFKLFNIQVKEVTQNDGTTTIANNLTSTVQVFTDSEYQLPYVLGSAHQGCLPPFPADVFMVPQYGYLTLNNGSQAVGRSSFYCLEYFPSQMLRTGNNFTFSYTFEDVPFHSSYAHSQSLDRLMNPLIDQYLYYLSRTNTPSGTTTQSRLQFSQAGASDIRDQSRNWLPGPCYRQQRVSKTSADNNNSEYSWTGATKYHLNGRDSLVNPGPAMASHKDDEEKFFPQSGVLIFGKQGSEKTNVDIEKVMITDEEEIRTTNPVATEQYGSVSTNLQRGNLAHPDTTKNARQAATADVNTQGVLPGMVWQDRDVYLQGPIWAKIPHTDGHFHPSPLMGGFGLKHPPPQILIKNTPVPANPSTTFSAAKFASFITQYSTGQVSVEIEWELQKENSKRWNPEIQYTSNYNKSVNVDFTVDTNGVYSEPRPIGTRYLTRNL

SEQ ID NO: 58 - protein, 737 aa, synthetic construct
  REGION 1..737: note = Ancestral capsid protein
  SITE 264: note = misc_feature - Xaa can be any naturally occurring amino acid
  SITE 266: note = misc_feature - Xaa can be any naturally occurring amino acid
  SITE 268: note = misc_feature - Xaa can be any naturally occurring amino acid
  SITE 448: note = misc_feature - Xaa can be any naturally occurring amino acid
  REGION 459..460: note = misc_feature - Xaa can be any naturally occurring amino acid
  SITE 467: note = misc_feature - Xaa can be any naturally occurring amino acid
  REGION 470..471: note = misc_feature - Xaa can be any naturally occurring amino acid
  SITE 474: note = misc_feature - Xaa can be any naturally occurring amino acid
  SITE 495: note = misc_feature - Xaa can be any naturally occurring amino acid
  SITE 516: note = misc_feature - Xaa can be any naturally occurring amino acid
  SITE 533: note = misc_feature - Xaa can be any naturally occurring amino acid
  SITE 547: note = misc_feature - Xaa can be any naturally occurring amino acid
  SITE 551: note = misc_feature - Xaa can be any naturally occurring amino acid
  SITE 555: note = misc_feature - Xaa can be any naturally occurring amino acid
  SITE 557: note = misc_feature - Xaa can be any naturally occurring amino acid
  SITE 561: note = misc_feature - Xaa can be any naturally occurring amino acid
  SITE 563: note = misc_feature - Xaa can be any naturally occurring amino acid
  SITE 577: note = misc_feature - Xaa can be any naturally occurring amino acid
  SITE 583: note = misc_feature - Xaa can be any naturally occurring amino acid
  SITE 593: note = misc_feature - Xaa can be any naturally occurring amino acid
  SITE 596: note = misc_feature - Xaa can be any naturally occurring amino acid
  REGION 661..662: note = misc_feature - Xaa can be any naturally occurring amino acid
  REGION 664..665: note = misc_feature - Xaa can be any naturally occurring amino acid
  SITE 710: note = misc_feature - Xaa can be any naturally occurring amino acid
  REGION 717..719: note = misc_feature - Xaa can be any naturally occurring amino acid
  SITE 723: note = misc_feature - Xaa can be any naturally occurring amino acid
MAADGYLPDWLEDNLSEGIREWWDLKPGAPKPKANQQKQDDGRGLVLPGYKYLGPFNGLDKGEPVNAADAAALEHDKAYDQQLKAGDNPYLRYNHADAEFQERLQEDTSFGGNLGRAVFQAKKRVLEPLGLVEEGAKTAPGKKRPVEPSPQRSPDSSTGIGKKGQQPAKKRLNFGQTGDSESVPDPQPLGEPPAGPSGLGSGTMAAGGGAPMADNNEGADGVGNASGNWHCDSTWLGDRVITTSTRTWALPTYNNHLYKQISSXSXGXTNDNHYFGYSTPWGYFDFNRFHCHFSPRDWQRLINNNWGFRPKRLNFKLFNIQVKEVTTNDGVTTIANNLTSTVQVFSDSEYQLPYVLGSAHQGCLPPFPADVFMIPQYGYLTLNNGSQAVGRSSFYCLEYFPSQMLRTGNNFTFSYTFEDVPFHSSYAHSQSLDRLMNPLIDQYLYYLXRTQSTGGTAGXXELLFSQXGPXXMSXQAKNWLPGPCYRQQRVSKTLXQNNNSNFAWTGATKYHLNGRXSLVNPGVAMATHKDDEXRFFPSSGVLIFGKXGAGXNNTXLXNVMXTXEEEIKTTNPVATEXYGVVAXNLQSSNTAPXTGXVNSQGALPGMVWQNRDVYLQGPIWAKIPHTDGNFHPSPLMGGFGLKHPPPQILIKNTPVPANPPXXFXXAKFASFITQYSTGQVSVEIEWELQKENSKRWNPEIQYTSNYAKSXNVDFAVXXXGVYXEPRPIGTRYLTRNL

SEQ ID NO: 59 - protein, 737 aa, synthetic construct
  REGION 1..737: note = Ancestral variant capsid
MAADGYLPDWLEDNLSEGIREWWDLKPGAPKPKANQQKQDDGRGLVLPGYKYLGPFNGLDKGEPVNAADAAALEHDKAYDQQLKAGDNPYLRYNHADAEFQERLQEDTSFGGNLGRAVFQAKKRVLEPLGLVEEGAKTAPGKKRPVEPSPQRSPDSSTGIGKKGQQPAKKRLNFGQTGDSESVPDPQPLGEPPAGPSGLGSGTMAAGGGAPMADNNEGADGVGNASGNWHCDSTWLGDRVITTSTRTWALPTYNNHLYKQISSASAGSTNDNHYFGYSTPWGYFDFNRFHCHFSPRDWQRLINNNWGFRPKRLNFKLFNIQVKEVTTNDGVTTIANNLTSTVQVFSDSEYQLPYVLGSAHQGCLPPFPADVFMIPQYGYLTLNNGSQAVGRSSFYCLEYFPSQMLRTGNNFTFSYTFEDVPFHSSYAHSQSLDRLMNPLIDQYLYYLARTQSTGGTAGTRELLFSQAGPSNMSAQAKNWLPGPCYRQQRVSKTLSQNNNSNFAWTGATKYHLNGRDSLVNPGVAMATHKDDEDRFFPSSGVLIFGKQGAGANNTALENVMMTSEEEIKTTNPVATEQYGVVASNLQSSNTAPVTGTVNSQGALPGMVWQNRDVYLQGPIWAKIPHTDGNFHPSPLMGGFGLKHPPPQILIKNTPVPANPPAVFTPAKFASFITQYSTGQVSVEIEWELQKENSKRWNPEIQYTSNYAKSTNVDFAVDNEGVYSEPRPIGTRYLTRNL

SEQ ID NO: 60 - protein, 10 aa, synthetic construct
  REGION 1..10: note = Heterologous peptide insertion
IAHDITKNIA

SEQ ID NO: 61 - protein, 7 aa, synthetic construct
  REGION 1..7: note = Heterologous peptide insertion
DITKNIA

SEQ ID NO: 62 - protein, 8 aa, synthetic construct
  REGION 1..8: note = Heterologous peptide insertion
NKTTNKDA

SEQ ID NO: 63 - protein, 8 aa, synthetic construct
  REGION 1..8: note = Heterologous peptide insertion
PQANANEN

SEQ ID NO: 64 - protein, 8 aa, synthetic construct
  REGION 1..8: note = Heterologous peptide insertion
PISNENEH